European Patent Specification EP 4 126 932 B1, published November 15, 2023. Title: Anti-BK virus antibody molecules. Applicant: Memo Therapeutics AG Universität Zürich Prorektorat Forschung Universität Bern Verwaltungsdirektion. The sequence listing filed with the application follows.

SEQUENCE LISTING (55 sequences)

SEQ ID NO: 1 - protein, 270 aa, Human polyomavirus 1
GGVEVLEVKTGVDAITEVECFLNPEMGDPDENLRGFSLKLSAENDFSSDSPERKMLPCYSTARIPLPNLNEDLTCGNLLMWEAVTVQTEVIGITSMLNLHAGSQKVHEHGGGKPIQGSNFHFFAVGGDPLEMQGVLMNYRTKYPDGTITPKNPTAQSQVMNTDHKAYLDKNNAYPVECWVPDPSRNENTRYFGTFTGGENVPPVLHVTNTATTVLLDEQGVGPLCKADSLYVSAADICGLFTNSSGTQQWRGLARYFKIRLRKRSVKNPY

SEQ ID NO: 2 - protein, 362 aa, Artificial Sequence
  BK pseudovirus, VP1-Ia
MAPTKRKGECPGAAPKKPKEPVQVPKLLIKGGVEVLEVKTGVDAITEVECFLNPEMGDPDENLRGFSLKLSAENDFSSDSPERKMLPCYSTARIPLPNLNEDLTCGNLLMWEAVTVQTEVIGITSMLNLHAGSQKVHEHGGGKPIQGSNFHFFAVGGDPLEMQGVLMNYRTKYPDGTITPKNPTAQSQVMNTDHKAYLDKNNAYPVECWVPDPSRNENTRYFGTFTGGENVPPVLHVTNTATTVLLDEQGVGPLCKADSLYVSAADICGLFTNSSGTQQWRGLARYFKIRLRKRSVKNPYPISFLLSDLINRRTQRVDGQPMYGMESQVEEVRVFDGTERLPGDPDMIRYIDKQGQLQTKML

SEQ ID NO: 3 - protein, 362 aa, Artificial Sequence
  BK pseudovirus, VP1-Ib
MAPTKRKGECPGAAPKKPKEPVQVPKLLIKGGVEVLEVKTGLDAITEVECFLNPEMGDPDENLRGFSLKLSAENDFSSDSPDRKMLPCYSTARIPLPNLNEDLTCGNLLMWEAVTVQTEVIGITSMLNLHAGSQKVHEHGGGKPIQGSNFHFFAVGGDPLEMQGVLMNYRTKYPEGTITPKNPTAQSQVMNTDHKAYLDKNNAYPVECWIPDPSRNENTRYFGTFTGGENVPPVLHVTNTATTVLLDEQGVGPLCKADSLYVSAADICGLFTNSSGTQQWRGLARYFKIRLRKRSVKNPYPISFLLSDLINRRTQRVDGQPMYGMESQVEEVRVFDGTERLPGDPDMIRYIDKQGQLQTKML

SEQ ID NO: 4 - protein, 270 aa, Human polyomavirus 1
GGVEVLEVKTGVDAITEVECFLNPEMGDPDDNLRGYSLKLTAENAFDSDSPDKKMLPCYSTARIPLPNLNEDLTCGNLLMWEAVTVKTEVIGITSMLNLHAGSQKVHENGGGKPVQGSNFHFFAVGGDPLEMQGVLMNYRTKYPQGTITPKNPTAQSQVMNTDHKAYLDKNNAYPVECWIPDPSRNENTRYFGTYTGGENVPPVLHVTNTATTVLLDEQGVGPLCKADSLYVSAADICGLFTNSSGTQQWRGLARYFKIRLRKRSVKNPY

SEQ ID NO: 5 - protein, 362 aa, Artificial Sequence
  BK pseudovirus, VP1-II
MAPTKRKGECPGAAPKKPKEPVQVPKLLIKGGVEVLEVKTGVDAITEVECFLNPEMGDPDDNLRGYSLKLTAENAFDSDSPDKKMLPCYSTARIPLPNLNEDLTCGNLLMWEAVTVKTEVIGITSMLNLHAGSQKVHENGGGKPVQGSNFHFFAVGGDPLEMQGVLMNYRTKYPQGTITPKNPTAQSQVMNTDHKAYLDKNNAYPVECWIPDPSRNENTRYFGTYTGGENVPPVLHVTNTATTVLLDEQGVGPLCKADSLYVSAADICGLFTNSSGTQQWRGLARYFKIRLRKRSVKNPYPISFLLSDLINRRTQRVDGQPMYGMESQVEEVRVFDGTEQLPGDPDMIRYIDRQGQLQTKMV

SEQ ID NO: 6 - protein, 362 aa, Human polyomavirus 1
MAPTKRKGECPGAAPKKPKEPVQVPKLLIKGGVEVLEVKTGVDAITEVECFLNPEMGDPDDNLRGYSQHLSAENAFESDSPDRKMLPCYSTARIPLPNLNEDLTCGNLLMWEAVTVKTEVIGITSMLNLHAGSQKVHENGGGKPVQGSNFHFFAVGGDPLEMQGVLMNYRTKYPQGTITPKNPTAQSQVMNTDHKAYLDKNNAYPVECWIPDPSRNENTRYFGTYTGGENVPPVLHVTNTATTVLLDEQGVGPLCKADSLYVSAADICGLFTNSSGTQQWRGLARYFKIRLRKRSVKNPYPISFLLSDLINRRTQKVDGQPMYGMESQVEEVRVFDGTEQLPGDPDMIRYIDRQGQLQTKMV

SEQ ID NO: 7 - protein, 362 aa, Artificial Sequence
  BK pseudovirus, VP1-III
MAPTKRKGECPGAAPKKPKEPVQVPKLLIKGGVEVLEVKTGVDAITEVECFLNPEMGDPDDNLRGYSQHLSAENAFESDSPDRKMLPCYSTARIPLPNLNEDLTCGNLLMWEAVTVKTEVIGITSMLNLHAGSQKVHENGGGKPVQGSNFHFFAVGGDPLEMQGVLMNYRTKYPQGTITPKNPTAQSQVMNTDHKAYLDKNNAYPVECWIPDPSRNENTRYFGTYTGGENVPPVLHVTNTATTVLLDEQGVGPLCKADSLYVSAADICGLFTNSSGTQQWRGLARYFKIRLRKRSVKNPYPISFLLSDLINRRTQRVDGQPMYGMESQVEEVRVFDGTEQLPGDPDMIRYIDRQGQLQTKMV

SEQ ID NO: 8 - protein, 270 aa, Human polyomavirus 1
GGVEVLEVKTGVDAITEVECFLNPEMGDPDNDLRGYSLRLTAETAFDSDSPDRKMLPCYSTARIPLPNLNEDLTCGNLLMWEAVTVKTEVIGITSMLNLHAGSQKVHENGGGKPIQGSNFHFFAVGGDPLEMQGVLMNYRTKYPEGTVTPKNPTAQSQVMNTDHKAYLDKNNAYPVECWIPDPSRNENTRYFGTYTGGENVPPVLHVTNTATTVLLDEQGVGPLCKADSLYVSAADICGLFTNSSGTQQWRGLPRYFKIRMRKRSVKNPY

SEQ ID NO: 9 - protein, 362 aa, Artificial Sequence
  BK pseudovirus, VP1-IVc
MAPTKRKGECPGAAPKKPKEPVQVPKLLIKGGVEVLEVKTGVDAITEVECFLNPEMGDPDNDLRGYSLRLTAETAFDSDSPDRKMLPCYSTARIPLPNLNEDLTCGNLLMWEAVTVKTEVIGITSMLNLHAGSQKVHENGGGKPIQGSNFHFFAVGGDPLEMQGVLMNYRTKYPEGTVTPKNPTAQSQVMNTDHKAYLDKNNAYPVECWIPDPSKNENTRYFGTYTGGENVPPVLHVTNTATTVLLDEQGVGPLCKADSLYVSAADICGLFTNSSGTQQWRGLPRYFKIRLRKRSVKNPYPISFLLSDLINRRTQRVDGQPMYGMESQVEEVRVFDGTEQLPGDPDMIRYIDRQGQLQTKMV

SEQ ID NO: 10 - protein, 270 aa, JC polyomavirus
GGVEVLEVKTGVDSITEVECFLTPEMGDPDEHLRGFSKSISISDTFESDSPNRDMLPCYSVARIPLPNLNEDLTCGNILMWEAVTLKTEVIGVTSLMNVHSNGQATHDNGAGKPVQGTSFHFFSVGGEALELQGVLFNYRTKYPDGTIFPKNATVQSQVMNTEHKAYLDKNKAYPVECWVPDPTRNENTRYFGTLTGGENVPPVLHITNTATTVLLDEFGVGPLCKGDNLYLSAVDVCGMFTNRSGSQQWRGLSRYFKVQLRKRRVKNPY

SEQ ID NO: 11 - protein, 5 aa, Artificial Sequence
  heavy chain complementarity determining region 1
NYWMT

SEQ ID NO: 12 - protein, 17 aa, Artificial Sequence
  heavy chain complementarity determining region 2
NIKKDGSEKYYVDSVRG

SEQ ID NO: 13 - protein, 11 aa, Artificial Sequence
  heavy chain complementarity determining region 3
VRSGRYFALDD

SEQ ID NO: 14 - protein, 11 aa, Artificial Sequence
  light chain complementarity determining region 1
GGDNIGSRPVH

SEQ ID NO: 15 - protein, 7 aa, Artificial Sequence
  light chain complementarity determining region 2
DDSNRPS

SEQ ID NO: 16 - protein, 10 aa, Artificial Sequence
  light chain complementarity determining region 3
QVWSSSTDHP

SEQ ID NO: 17 - protein, 120 aa, Artificial Sequence
  heavy chain variable region
QVQLVESGGTLVQPGGSLRLSCAASGFTFNNYWMTWVRQAPGKGLEWVANIKKDGSEKYYVDSVRGRFTISRDNAKNSLFLQMNSLRPEDTAVYFCATVRSGRYFALDDWGQGTLVTVSS

SEQ ID NO: 18 - protein, 107 aa, Artificial Sequence
  light chain variable region
QSVLTQPPSVSVAPGKTARITCGGDNIGSRPVHWYQQKPGQAPILVVYDDSNRPSGIPERFSGSNSGNTATLTISRVEAGDEADYYCQVWSSSTDHPFGGGTKVTVL

SEQ ID NO: 19 - protein, 450 aa, Artificial Sequence
  full length heavy chain
QVQLVESGGTLVQPGGSLRLSCAASGFTFNNYWMTWVRQAPGKGLEWVANIKKDGSEKYYVDSVRGRFTISRDNAKNSLFLQMNSLRPEDTAVYFCATVRSGRYFALDDWGQGTLVTVSSASTKGPSVFPLAPSSKSTSGGTAALGCLVKDYFPEPVTVSWNSGALTSGVHTFPAVLQSSGLYSLSSVVTVPSSSLGTQTYICNVNHKPSNTKVDKKVEPKSCDKTHTCPPCPAPELLGGPSVFLFPPKPKDTLMISRTPEVTCVVVDVSHEDPEVKFNWYVDGVEVHNAKTKPREEQYNSTYRVVSVLTVLHQDWLNGKEYKCKVSNKALPAPIEKTISKAKGQPREPQVYTLPPSREEMTKNQVSLTCLVKGFYPSDIAVEWESNGQPENNYKTTPPVLDSDGSFFLYSKLTVDKSRWQQGNVFSCSVMHEALHNHYTQKSLSLSPGK

SEQ ID NO: 20 - protein, 213 aa, Artificial Sequence
  full length light chain
QSVLTQPPSVSVAPGKTARITCGGDNIGSRPVHWYQQKPGQAPILVVYDDSNRPSGIPERFSGSNSGNTATLTISRVEAGDEADYYCQVWSSSTDHPFGGGTKVTVLGQPKAAPSVTLFPPSSEELQANKATLVCLISDFYPGAVTVAWKADSSPVKAGVETTTPSKQSNNKYAASSYLSLTPEQWKSHRSYSCQVTHEGSTVEKTVAPTECS

SEQ ID NO: 21 - protein, 5 aa, Artificial Sequence
  heavy chain complementarity determining region 1
AYYWT

SEQ ID NO: 22 - protein, 16 aa, Artificial Sequence
  heavy chain complementarity determining region 2
EINHRGYTNYNPSLRG

SEQ ID NO: 23 - protein, 13 aa, Artificial Sequence
  heavy chain complementarity determining region 3
LRSTSGWHDYFDY

SEQ ID NO: 24 - protein, 12 aa, Artificial Sequence
  light chain complementarity determining region 1
RASQSVSSSYLA

SEQ ID NO: 25 - protein, 7 aa, Artificial Sequence
  light chain complementarity determining region 2
GASSRAT

SEQ ID NO: 26 - protein, 9 aa, Artificial Sequence
  light chain complementarity determining region 3
LQYGSSPLT

SEQ ID NO: 27 - protein, 121 aa, Artificial Sequence
  heavy chain variable region
QVQLQQWGAGLLKPSETLSLTCAVYRGSFSAYYWTWFRQPPGKGLEWIGEINHRGYTNYNPSLRGRVSISVDTSKKQFSLKLRSVNAADTAVYYCATLRSTSGWHDYFDYWGQGTLVTVSS

SEQ ID NO: 28 - protein, 108 aa, Artificial Sequence
  light chain variable region
EIVLTQSPGTLSLSPGERATLSCRASQSVSSSYLAWYQQTPGQAPRLLIYGASSRATGIPDRFSGSGSGTDFTLTISRLEPEDFVVYFCLQYGSSPLTFGPGTKVDIK

SEQ ID NO: 29 - protein, 451 aa, Artificial Sequence
  full length heavy chain
QVQLQQWGAGLLKPSETLSLTCAVYRGSFSAYYWTWFRQPPGKGLEWIGEINHRGYTNYNPSLRGRVSISVDTSKKQFSLKLRSVNAADTAVYYCATLRSTSGWHDYFDYWGQGTLVTVSSASTKGPSVFPLAPSSKSTSGGTAALGCLVKDYFPEPVTVSWNSGALTSGVHTFPAVLQSSGLYSLSSVVTVPSSSLGTQTYICNVNHKPSNTKVDKKVEPKSCDKTHTCPPCPAPELLGGPSVFLFPPKPKDTLMISRTPEVTCVVVDVSHEDPEVKFNWYVDGVEVHNAKTKPREEQYNSTYRVVSVLTVLHQDWLNGKEYKCKVSNKALPAPIEKTISKAKGQPREPQVYTLPPSREEMTKNQVSLTCLVKGFYPSDIAVEWESNGQPENNYKTTPPVLDSDGSFFLYSKLTVDKSRWQQGNVFSCSVMHEALHNHYTQKSLSLSPGK

SEQ ID NO: 30 - protein, 215 aa, Artificial Sequence
  full length light chain
EIVLTQSPGTLSLSPGERATLSCRASQSVSSSYLAWYQQTPGQAPRLLIYGASSRATGIPDRFSGSGSGTDFTLTISRLEPEDFVVYFCLQYGSSPLTFGPGTKVDIKRTVAAPSVFIFPPSDEQLKSGTASVVCLLNNFYPREAKVQWKVDNALQSGNSQESVTEQDSKDSTYSLSSTLTLSKADYEKHKVYACEVTHQGLSSPVTKSFNRGEC

SEQ ID NO: 31 - protein, 108 aa, Artificial Sequence
  light chain variable region
EIVLTQSPGTLSLSPGERATLSCRASQSVSSSYLAWYQQKPGQAPRLLIYGASSRATGIPDRFSGSGSGTDFTLTISRLEPEDFAVYFCLQYGSSPLTFGPGTKVDIK

SEQ ID NO: 32 - protein, 451 aa, Artificial Sequence; identical to SEQ ID NO: 29
  full length heavy chain

SEQ ID NO: 33 - protein, 215 aa, Artificial Sequence
  full length light chain
EIVLTQSPGTLSLSPGERATLSCRASQSVSSSYLAWYQQKPGQAPRLLIYGASSRATGIPDRFSGSGSGTDFTLTISRLEPEDFAVYFCLQYGSSPLTFGPGTKVDIKRTVAAPSVFIFPPSDEQLKSGTASVVCLLNNFYPREAKVQWKVDNALQSGNSQESVTEQDSKDSTYSLSSTLTLSKADYEKHKVYACEVTHQGLSSPVTKSFNRGEC

SEQ ID NO: 34 - protein, 5 aa, Artificial Sequence
  heavy chain complementarity determining region 1
LYAMN

SEQ ID NO: 35 - protein, 17 aa, Artificial Sequence
  heavy chain complementarity determining region 2
LISGSGTATYYADSVTG

SEQ ID NO: 36 - protein, 15 aa, Artificial Sequence
  heavy chain complementarity determining region 3
TYPTWGGVVIGAIDV

SEQ ID NO: 37 - protein, 11 aa, Artificial Sequence
  light chain complementarity determining region 1
RASQSIQRWLA

SEQ ID NO: 38 - protein, 7 aa, Artificial Sequence
  light chain complementarity determining region 2
DASTLES

SEQ ID NO: 39 - protein, 9 aa, Artificial Sequence
  light chain complementarity determining region 3
QQYNGHAST

SEQ ID NO: 40 - protein, 124 aa, Artificial Sequence
  heavy chain variable region
EEPLLESGGGLVQPGGSLRLSCAASGFTFRLYAMNWVRQAPGKGLEWVSLISGSGTATYYADSVTGRFSISRDNYKNRVYLQMDSLRADDTATYYCAKTYPTWGGVVIGAIDVWGQGTTVTVSS

SEQ ID NO: 41 - protein, 107 aa, Artificial Sequence
  light chain variable region
DIQMTQSPSTLSASVGDRVTITCRASQSIQRWLAWHQQKPGRAPKVLIHDASTLESGVPSRFSGSGSGTEFTLTISSLQPDDFATYYCQQYNGHASTFGPGTKVDIK

SEQ ID NO: 42 - protein, 454 aa, Artificial Sequence
  full length heavy chain
EEPLLESGGGLVQPGGSLRLSCAASGFTFRLYAMNWVRQAPGKGLEWVSLISGSGTATYYADSVTGRFSISRDNYKNRVYLQMDSLRADDTATYYCAKTYPTWGGVVIGAIDVWGQGTTVTVSSASTKGPSVFPLAPSSKSTSGGTAALGCLVKDYFPEPVTVSWNSGALTSGVHTFPAVLQSSGLYSLSSVVTVPSSSLGTQTYICNVNHKPSNTKVDKKVEPKSCDKTHTCPPCPAPELLGGPSVFLFPPKPKDTLMISRTPEVTCVVVDVSHEDPEVKFNWYVDGVEVHNAKTKPREEQYNSTYRVVSVLTVLHQDWLNGKEYKCKVSNKALPAPIEKTISKAKGQPREPQVYTLPPSREEMTKNQVSLTCLVKGFYPSDIAVEWESNGQPENNYKTTPPVLDSDGSFFLYSKLTVDKSRWQQGNVFSCSVMHEALHNHYTQKSLSLSPGK

SEQ ID NO: 43 - protein, 214 aa, Artificial Sequence
  full length light chain
DIQMTQSPSTLSASVGDRVTITCRASQSIQRWLAWHQQKPGRAPKVLIHDASTLESGVPSRFSGSGSGTEFTLTISSLQPDDFATYYCQQYNGHASTFGPGTKVDIKRTVAAPSVFIFPPSDEQLKSGTASVVCLLNNFYPREAKVQWKVDNALQSGNSQESVTEQDSKDSTYSLSSTLTLSKADYEKHKVYACEVTHQGLSSPVTKSFNRGEC

SEQ ID NO: 44 - protein, 17 aa, Artificial Sequence
  heavy chain complementarity determining region 2
LISGSGTATYYADSVKG

SEQ ID NO: 45 - protein, 124 aa, Artificial Sequence
  heavy chain variable region
EEPLLESGGGLVQPGGSLRLSCAASGFTFRLYAMNWVRQAPGKGLEWVSLISGSGTATYYADSVKGRFSISRDNSKNRVYLQMSSLRADDTATYYCAKTYPTWGGVVIGAIDVWGQGTTVTVSS

SEQ ID NO: 46 - protein, 454 aa, Artificial Sequence
  full length heavy chain
EEPLLESGGGLVQPGGSLRLSCAASGFTFRLYAMNWVRQAPGKGLEWVSLISGSGTATYYADSVKGRFSISRDNSKNRVYLQMSSLRADDTATYYCAKTYPTWGGVVIGAIDVWGQGTTVTVSSASTKGPSVFPLAPSSKSTSGGTAALGCLVKDYFPEPVTVSWNSGALTSGVHTFPAVLQSSGLYSLSSVVTVPSSSLGTQTYICNVNHKPSNTKVDKKVEPKSCDKTHTCPPCPAPELLGGPSVFLFPPKPKDTLMISRTPEVTCVVVDVSHEDPEVKFNWYVDGVEVHNAKTKPREEQYNSTYRVVSVLTVLHQDWLNGKEYKCKVSNKALPAPIEKTISKAKGQPREPQVYTLPPSREEMTKNQVSLTCLVKGFYPSDIAVEWESNGQPENNYKTTPPVLDSDGSFFLYSKLTVDKSRWQQGNVFSCSVMHEALHNHYTQKSLSLSPGK

SEQ ID NO: 47 - protein, 214 aa, Artificial Sequence; identical to SEQ ID NO: 43
  full length light chain

SEQ ID NO: 48 - protein, 9 aa, Artificial Sequence
  light chain complementarity determining region 3
QQYSGHAST

SEQ ID NO: 49 - protein, 124 aa, Artificial Sequence
  heavy chain variable region
EEPLLESGGGLVQPGGSLRLSCAASGFTFRLYAMNWVRQAPGKGLEWVSLISGSGTATYYADSVKGRFTISRDNSKNRVYLQMSSLRADDTAVYYCAKTYPTWGGVVIGAIDVWGQGTTVTVSS

SEQ ID NO: 50 - protein, 107 aa, Artificial Sequence
  light chain variable region
DIQMTQSPSTLSASVGDRVTITCRASQSIQRWLAWHQQKPGKAPKLLIHDASTLESGVPSRFSGSGSGTEFTLTISSLQPDDFATYYCQQYSGHASTFGPGTKVDIK

SEQ ID NO: 51 - protein, 454 aa, Artificial Sequence
  full length heavy chain
EEPLLESGGGLVQPGGSLRLSCAASGFTFRLYAMNWVRQAPGKGLEWVSLISGSGTATYYADSVKGRFTISRDNSKNRVYLQMSSLRADDTAVYYCAKTYPTWGGVVIGAIDVWGQGTTVTVSSASTKGPSVFPLAPSSKSTSGGTAALGCLVKDYFPEPVTVSWNSGALTSGVHTFPAVLQSSGLYSLSSVVTVPSSSLGTQTYICNVNHKPSNTKVDKKVEPKSCDKTHTCPPCPAPELLGGPSVFLFPPKPKDTLMISRTPEVTCVVVDVSHEDPEVKFNWYVDGVEVHNAKTKPREEQYNSTYRVVSVLTVLHQDWLNGKEYKCKVSNKALPAPIEKTISKAKGQPREPQVYTLPPSREEMTKNQVSLTCLVKGFYPSDIAVEWESNGQPENNYKTTPPVLDSDGSFFLYSKLTVDKSRWQQGNVFSCSVMHEALHNHYTQKSLSLSPGK

SEQ ID NO: 52 - protein, 214 aa, Artificial Sequence
  full length light chain
DIQMTQSPSTLSASVGDRVTITCRASQSIQRWLAWHQQKPGKAPKLLIHDASTLESGVPSRFSGSGSGTEFTLTISSLQPDDFATYYCQQYSGHASTFGPGTKVDIKRTVAAPSVFIFPPSDEQLKSGTASVVCLLNNFYPREAKVQWKVDNALQSGNSQESVTEQDSKDSTYSLSSTLTLSKADYEKHKVYACEVTHQGLSSPVTKSFNRGEC

SEQ ID NO: 53 - DNA, 20 bp, Artificial Sequence
  qPCR primer
ggatgggcagcctatgtatg

SEQ ID NO: 54 - DNA, 20 bp, Artificial Sequence
  qPCR primer
tcatatctgggtcccctgga

SEQ ID NO: 55 - DNA, 20 bp, Artificial Sequence
  qPCR probe
agggtgtttgatggcacaga